European Patent Application EP 4 800 100 A1, published September 2, 2026. Title: 溶瘤病毒及其用途. Applicant: 上海元宋生物技术有限公司. The sequence listing filed with the application follows.

SEQUENCE LISTING (4 sequences)

SEQ ID NO: 1 - DNA, 573 bp, synthetic construct
  source 1..573: mol_type = other DNA
atggccctgtccttcagcctgctgatggccgtgctggtgctgagctacaagtccatctgctccctgggcatgtgtgatctgcctcagacacactccctgggcaatagaagggccctgatcctgctggcccagatgagaaggatcagccccttctcctgcctgaaggatagacacgattttggcttccctcaggaggagttcgacggcaatcagtttcagaaggcccaggccatctccgtgctgcacgagatgatccagcagacctttaacctgttctccacaaaggactccagcgccgcctgggacgagtccctgctggagaagttttacacagagctgtaccagcagctgaacgatctggaggcctgcgtgatccaggaggtgggcgtggaggagacccccctgatgaatgtggattccatcctggccgtgaagaagtactttcagagaatcaccctgtacctgaccgagaagaagtacagcccttgtgcctgggaggtggtgagagccgagatcatgagatccttttccctgagcacaaacctgcaggagaggctgagaaggaaggagtga

SEQ ID NO: 2 - DNA, 573 bp, synthetic construct
  source 1..573: mol_type = other DNA
atggccctgtccttctccctgctgatggccgtgctggtgctgagctacaagtccatctgctccctgggcatgtgcgacctgcctcagacacactccctgggcaataggagagccctgatcctgctggcccagatgaggaggatctccccttttagctgcctgaaggatagacacgatttcggcttccctcaggaggagttcgatggcaatcagttccagaaggcccaggccatcagcgtgctgcacgagatgatccagcagaccttcaatctgtttagcaccaaggactccagcgccgcctgggacgagtccctgctggagaagttctacaccgagctgtaccagcagctgaacgacctggaggcctgcgtgatccaggaggtgggcgtggaggagacccctctgatgaatgtggatagcatcctggccgtgaagaagtactttcagagaatcacactgtacctgacagagaagaagtacagcccctgcgcctgggaggtggtgagggctgagatcatgaggagcttttccctgtccacaaacctgcaggagaggctgagaaggaaggagtga

SEQ ID NO: 3 - DNA, 573 bp, synthetic construct
  source 1..573: mol_type = other DNA
atggccctgtccttttctttactgatggccgtgctggtgctcagctacaaatccatctgttctctgggcatgtgcgacctgccgcagacccactccctgggtaaccgtcgtgctctgatcctgctggctcagatgcgtcgtatctccccgttctcctgcctgaaagaccgtcacgacttcggtttcccgcaggaagaattcgacggtaaccagttccagaaagctcaggctatctccgttctgcacgaaatgatccagcagaccttcaacctgttctccaccaaagactcctccgctgcttgggacgaatccctgctggaaaaattctacaccgaactgtaccagcagctgaacgacctggaagcttgcgttatccaggaagttggtgttgaagaaaccccgctgatgaacgttgactccatcctggctgttaaaaaatacttccagcgtatcaccctgtacctgaccgaaaaaaaatactccccgtgcgcttgggaagttgttcgtgctgaaatcatgcgttccttctccctgtccaccaacctgcaggaacgtctgcgtcgtaaagaataa

SEQ ID NO: 4 - protein, 167 aa, synthetic construct
MCDLPQTHSLGNRRALILLAQMRRISPFSCLKDRHDFGFPQEEFDGNQFQKAQAISVLHEMIQQTFNLFSTKDSSAAWDESLLEKFYTELYQQLNDLEACVIQEVGVEETPLMNVDSILAVKKYFQRITLYLTEKKYSPCAWEVVRAEIMRSFSLSTNLQERLRRKE